European Patent Application EP 4 763 862 A1, published June 24, 2026. Title: 结合B7-H3的抗体及其用途. Applicant: 北京泰德制药股份有限公司. The sequence listing filed with the application follows.

SEQUENCE LISTING (272 sequences)

SEQ ID NO: 1 - protein, 120 aa, synthetic construct
  REGION 1..120: note = VH
EVQLQQSGTELVRPGALVKLSCKTSGFNIKDCYMHWVKQRPEQGLEWIGWIDPENGNTIYDPKFQGKATITADTSSYTAYLQLSSLTSEDTAVYYCARSRARGYAMDYWGQGTSVTVTSS

SEQ ID NO: 2 - protein, 111 aa, synthetic construct
  REGION 1..111: note = VL
DIVMTQSPASLAVSLGQRATISCRASQSVSTSSYSYMHWYRQIPGQPPKLLIKYASNLESGVPARFSGSGSGTDFTLNIHPVEEEDTATYYCQHSWEIPRTFGGGTKLELK

SEQ ID NO: 3 - protein, 118 aa, synthetic construct
  REGION 1..118: note = VH
EVQLQESGGDLVKPGGSLKLSCAASGFTFSSYGMSWVRQTPEKRLEWVASISGSGSYTYYPDSLKGRFTISRDNAKNNLYLQMSSLRSEDTALYYCARQDGYWYFDVWGAGTTVTVSS

SEQ ID NO: 4 - protein, 107 aa, synthetic construct
  REGION 1..107: note = VL
DILMTQTPKFLLVSAGDRVTITCKASQSVSNDVAWYQQKPGQSPQLLIYYASHRYTGVPDRFTGSGYGTDFTFTISTVQAEDLAVYFCQQDNSSPLTFGAGTKLELK

SEQ ID NO: 5 - protein, 117 aa, synthetic construct
  REGION 1..117: note = VH
EVQVVESGPELVKPGASVKMSCKTSAYTFSDSVLSWVKQRTGQGLEWIGEIYPRGNVTHYNGKFKGKATLTADKSSNTAFMHFSSLTSEDSAVYFCARWNNFFFDYWGQGSTLTVSS

SEQ ID NO: 6 - protein, 112 aa, synthetic construct
  REGION 1..112: note = VL
DIVMTQPPLSLPVTLGDLASISCRSSQSLVHSNGITYLHWYLQKPGQSPKLLIYKVSNRFSGVPDRFSGSGSGTDFTLKISRVEAEDLGVYFCSQSTHFPWTFGGGTKLELK

SEQ ID NO: 7 - protein, 118 aa, synthetic construct
  REGION 1..118: note = VH
EVQLQQSGPSLVKPSQTLSLTCSVTGGSITSFYWNWIRKFPGNKLEYMGYISSSGSTYYNPSLKSRISITRDTSKNQSYLQLNSVTAEDTATYYCARGGVHYGFGDYWGQGTSVTVSS

SEQ ID NO: 8 - protein, 112 aa, synthetic construct
  REGION 1..112: note = VL
DIVMTQSAPSVPVTPGESVSISCRSSKSLLHSNGNTYLYWFLQRPGQSPQLLIYRMSNLASGVPDRFSGSGSGTAFTLRISRVEAEDVGVYYCMQHLEYPLTFGAGTKLELK

SEQ ID NO: 9 - protein, 120 aa, synthetic construct
  REGION 1..120: note = VH
EVQLVESGGGLVQPGGSLRVSCATSGFTFSDYYMSWVRQPPGKALEWLGFIRNKINGYTTEYSASVKGRFTISRDNSQSILYLQMNTLRAEDSATYYCTRDSSQRPFAYWGQGTLVTVSA

SEQ ID NO: 10 - protein, 113 aa, synthetic construct
  REGION 1..113: note = VL
DIVMTQSPSSLSVSAGEKVTMTCKSSQSLLNSRSQKNFLAWYQQKPGQPPKLLIYGASTRESGVPDRFTGSGSGTDFTLTISNVQAEDLAVYYCQNDLTYPLTFGAGTKLELK

SEQ ID NO: 11 - protein, 121 aa, synthetic construct
  REGION 1..121: note = VH
EVQLQQSGPELVRPGVSVKISCKGSGYTFTDYAMHWVKQSHAKSLEWIGVINTYSGNTYYSQKFKGKATMTVDKSSSTAYMELARLTSEDSAIYYCARGAGYFPYWYFDVWGAGTTVTVSS

SEQ ID NO: 12 - protein, 107 aa, synthetic construct
  REGION 1..107: note = VL
DIQMIQSPSYLAASPGETITINCRASKSISKYLAWYQEKPGKTNKLLIYSGSTLQSGIPSRFSGSGSGTDFTLTISSLEPEDFAMYYCQQHYEYPYTFGGGTKLEIK

SEQ ID NO: 13 - protein, 112 aa, synthetic construct
  REGION 1..112: note = VL
DVLMTQTPLSLPVSLGDQVSISCRASQSLANSYGKTYLSWYLHKPGQSPQLLIYGISNRFSGVPDRFSGSGSGTDFTLKISTIKPEDLGMYYCLHGTHQPLTFGAGTKLELK

SEQ ID NO: 14 - protein, 119 aa, synthetic construct
  REGION 1..119: note = VH
EVKLQESGPGLVKPSQSLSLTCTVTGYSITSDYAWNWIRQFPGNILEWMGYISYSGSASYNPSLQSRISVTRDTSKNQFFLQLNSVTTEDTATYYCVRSLGRRWYFGFWGAGTTVTVSS

SEQ ID NO: 15 - protein, 113 aa, synthetic construct
  REGION 1..113: note = VL
DIVLTQSPSSLAMTVGQKVTMSCKSSQNLLNSSNQKNYLAWYQQKPGQSPKLLVYFASTRESGVPDRFIGSGSGTDFTLTISSVQAEDLADYFCQQHYSTPLTFGGGTKLEIK

SEQ ID NO: 16 - protein, 119 aa, synthetic construct
  REGION 1..119: note = VH
EVQLVESGGGLVKPGGSLKLSCAVSGFTFSSYAMSWVRQTPEKRLEWVASITDGGITFYSDSLKGRFTISRDNSGNILYLQMSSLRSEDTAMYFCARGSITTDWYFDVWGAGTTVTVSS

SEQ ID NO: 17 - protein, 113 aa, synthetic construct
  REGION 1..113: note = VL
DIVMTQAPLSLPVSLGDQASISCRSSQSLVHSNGNTYLHWYLQKPGQSPKLLIYKVSNRFSGVPDRFSGSGSGTDFTLKISRVEAEDLGVYFCSQSTHVPPYTFGGGTKLEIK

SEQ ID NO: 18 - protein, 121 aa, synthetic construct
  REGION 1..121: note = VH
EVQLQQSGPELVRPGVSVKISCKGSGYTFTDYSMHWVKQSHAKSLEWIGVINTSSGNTYYNLKFKGKATMTVDKSSSTAYMELARLTSEDSAIYYCSKYYGSSFHWYFDVWGAGTTVTVSS

SEQ ID NO: 19 - protein, 106 aa, synthetic construct
  REGION 1..106: note = VL
DIVMTQSPVIMSASPGEKVTMTCSASSSVSYMHWYQQKSSTSPKLWIYDTSKLASGVPGRFSGTGSGKSHSLTISSMEAEDVATYYCFQGSGYPLTFGSGTKLEIK

SEQ ID NO: 20 - protein, 121 aa, synthetic construct
  REGION 1..121: note = VH
EVQLQQSGPELVRPGESVKISCKGSGYTFTDYAIHWVKQSHAKSLEWIGVISTYYDNTYYNQKFKGRATMTVDKSSSTAYMELARLTSEDSAIYYCARGYGSSFNWYFDVWGAGTTVTVSS

SEQ ID NO: 21 - protein, 112 aa, synthetic construct
  REGION 1..112: note = VL
DIVMTQSPSSLAVSAGEKVTMSCKSSQSLLNSRTRKNYLAWYQQKPGQSPKLLIYWASTRESGVPDRFTGSGSGTDFTLTITSVQAEDLAVYYCKQSYNLYTFGGGTKLEIK

SEQ ID NO: 22 - protein, 118 aa, synthetic construct
  REGION 1..118: note = VH
EVKLVESGAVLVKPGASVKISCKASGYTLSDFNMDWVKQSQGKSLEWVGDINPNYDTITYNQKFRGKATLTVDRSSNTAYMELRSLTSEDSAVYYCARGELGRYFYVWGAGTTVTVSS

SEQ ID NO: 23 - protein, 107 aa, synthetic construct
  REGION 1..107: note = VL
DIQLTQPPASLSASVGETVTITCRASENVYSYLAWYRQKQGRSPQLLVYNAKTLPEGVPSRFSGSGSGTQFSLKINSLQTEDLGDYYCQHHYGTPWTFGGGTKLEIK

SEQ ID NO: 24 - protein, 115 aa, synthetic construct
  REGION 1..115: note = VH
EVQLQQSGAELVQPGASMKLSCKTSGYTFTTYDINWVRQRPEQGLEWIGWIFPGDGTTKYNEKFKGKATLTTDKSSSTAYMHLSRLTSEDSVVYFCARTPWFDYWGQGTTLTVSS

SEQ ID NO: 25 - protein, 105 aa, synthetic construct
  REGION 1..105: note = VL
DIVLSQSPAIMSASPGEKVIMTCSASSSISYMYWYQQKPGTSPKRWIYDTSKLASGVPARFSVSGSGTSYSLTISSMEAEDAATYYCHQRSSYPTFGGGTKLELK

SEQ ID NO: 26 - protein, 118 aa, synthetic construct
  REGION 1..118: note = VH
EVQLVESGGGLVKPGGSLRLSCAASGFTFSSYGMSWVRQAPGKGLEWVSSISGSGSYTYYPDSLKGRFTISRDNAKNSLYLQMNSLRAEDTAVYYCARQQGYWYFDVWGQGTTVTVSS

SEQ ID NO: 27 - protein, 112 aa, synthetic construct
  REGION 1..112: note = VL
DIVMTQTPLSLPVTPGEPASISCRASQSLASSYGKTYLSWYLQKPGQSPQLLIYGISNRFSGVPDRFSGSGSGTDFTLKISRVEAEDVGVYYCLHGTHQPLTFGQGTKLEIK

SEQ ID NO: 28 - protein, 118 aa, synthetic construct
  REGION 1..118: note = VH
EVQLVESGGGLVKPGGSLRLSCAASGFTFSSYGMSWVRQAPGKRLEWVSSISGSGSYTYYPDSLKGRFTISRDNAKNSLYLQMNSLRAEDTAVYYCARQQGYWYFDVWGQGTTVTVSS

SEQ ID NO: 29 - protein, 112 aa, synthetic construct
  REGION 1..112: note = VL
DVVMTQTPLSLPVTPGEPASISCRASQSLASSYGKTYLSWYLQKPGQSPQLLIYGISNRFSGVPDRFSGSGSGTDFTLKISRVEAEDVGVYYCLHGTHQPLTFGQGTKLEIK

SEQ ID NO: 30 - protein, 118 aa, synthetic construct
  REGION 1..118: note = VH
EVQLVESGGGLVKPGGSLRLSCAASGFTFSSYGMSWVRQAPGKRLEWVASISGSGSYTYYPDSLKGRFTISRDNAKNSLYLQMNSLRAEDTAVYYCARQQGYWYFDVWGQGTTVTVSS

SEQ ID NO: 31 - protein, 118 aa, synthetic construct; identical to SEQ ID NO: 3
  REGION 1..118: note = VH

SEQ ID NO: 32 - protein, 112 aa, synthetic construct; identical to SEQ ID NO: 13
  REGION 1..112: note = VL

SEQ ID NO: 33 - protein, 118 aa, synthetic construct; identical to SEQ ID NO: 22
  REGION 1..118: note = VH

SEQ ID NO: 34 - protein, 118 aa, synthetic construct
  REGION 1..118: note = VH
QVQLVESGAVVKKPGASVKVSCKASGYTLSDFNMDWVRQAPGKSLEWMGDINPNYDTITYNQKFRGRVTLTVDRSINTAYMELSRLRSDDTAVYYCARGELGRYFYVWGAGTMVTVSS

SEQ ID NO: 35 - protein, 118 aa, synthetic construct
  REGION 1..118: note = VH
EVQLVESGAVVKKPGASVKVSCKASGYTLSDFNMDWVRQAPGKSLEWMGDINPNYDTITYNQKFRGRVTLTVDRSANTAYMELSSLRSEDTAVYYCARGELGRYFYVWGAGTMVTVSS

SEQ ID NO: 36 - protein, 118 aa, synthetic construct
  REGION 1..118: note = VH
EVKLVESGAEVKKPGASVKVSCKASGYTLSDFNMDWVRQAPGKSLEWMGDINPNYDTITYNQKFRGRVTLTVDRSTNTAYMELSSLRSEDTAVYYCARGELGRYFYVWGAGTMVTVSS

SEQ ID NO: 37 - protein, 118 aa, synthetic construct
  REGION 1..118: note = VH
QVQLVESGAEVKKPGASVKVSCKASGYTLSDFNMDWVRQAQGKSLEWMGDINPNYDTITYNQKFRGRVTLTVDRSTNTAYMELSSLRSEDTAVYYCARGELGRYFYVWGAGTMVTVSS

SEQ ID NO: 38 - protein, 107 aa, synthetic construct
  REGION 1..107: note = VL
DIQLTQPPSSLSASVGDRVTITCRASENVYSYLAWYQQKPGRSPQLLVYNAKTLQEGVPSRFSGSGSGTQFTLTISSLQPEDFADYYCQHHYGTPWTFGGGTKVEIK

SEQ ID NO: 39 - protein, 107 aa, synthetic construct; identical to SEQ ID NO: 38
  REGION 1..107: note = VL

SEQ ID NO: 40 - protein, 107 aa, synthetic construct
  REGION 1..107: note = VL
DIQLTQPPSFLSASVGDRVTITCRASENVYSYLAWYQQKPGRSPQLLVYNAKTLQEGVPSRFSGSGSGTEFTLTISSLQPEDFADYYCQHHYGTPWTFGGGTKVEIK

SEQ ID NO: 41 - protein, 107 aa, synthetic construct
  REGION 1..107: note = VL
DIQLTQPPSSLSASVGDRVTITCRASENVYSYLAWYQQKPGRSPQLLVYNAKTLQEGVPSRFSGSGSGTQFTLTISSLQPEDVADYYCQHHYGTPWTFGGGTKVEIK

SEQ ID NO: 42 - protein, 107 aa, synthetic construct
  REGION 1..107: note = VL
DIQLTQPPSSLSASVGDRVTITCRASENVYSYLAWYQQKPGRSPQLLVYNAKTLPEGVPSRFSGSGSGTQFTLTISSLQPEDFADYYCSHHYGTPWTFGGGTKVEIK

SEQ ID NO: 43 - protein, 25 aa, synthetic construct
  REGION 1..25: note = FR1
EVQLQQSGTELVRPGALVKLSCKTS

SEQ ID NO: 44 - protein, 7 aa, synthetic construct
  REGION 1..7: note = CDR1
GFNIKDC

SEQ ID NO: 45 - protein, 18 aa, synthetic construct
  REGION 1..18: note = FR2
YMHWVKQRPEQGLEWIGW

SEQ ID NO: 46 - protein, 8 aa, synthetic construct
  REGION 1..8: note = CDR2
IDPENGNT

SEQ ID NO: 47 - protein, 38 aa, synthetic construct
  REGION 1..38: note = FR3
IYDPKFQGKATITADTSSYTAYLQLSSLTSEDTAVYYC

SEQ ID NO: 48 - protein, 12 aa, synthetic construct
  REGION 1..12: note = CDR3
ARSRARGYAMDY

SEQ ID NO: 49 - protein, 12 aa, synthetic construct
  REGION 1..12: note = FR4
WGQGTSVTVTSS

SEQ ID NO: 50 - protein, 25 aa, synthetic construct
  REGION 1..25: note = FR1
EVQLQESGGDLVKPGGSLKLSCAAS

SEQ ID NO: 51 - protein, 7 aa, synthetic construct
  REGION 1..7: note = CDR1
GFTFSSY

SEQ ID NO: 52 - protein, 18 aa, synthetic construct
  REGION 1..18: note = FR2
GMSWVRQTPEKRLEWVAS

SEQ ID NO: 53 - protein, 8 aa, synthetic construct
  REGION 1..8: note = CDR2
ISGSGSYT

SEQ ID NO: 54 - protein, 38 aa, synthetic construct
  REGION 1..38: note = FR3
YYPDSLKGRFTISRDNAKNNLYLQMSSLRSEDTALYYC

SEQ ID NO: 55 - protein, 11 aa, synthetic construct
  REGION 1..11: note = CDR3
ARQDGYWYFDV

SEQ ID NO: 56 - protein, 11 aa, synthetic construct
  REGION 1..11: note = FR4
WGAGTTVTVSS

SEQ ID NO: 57 - protein, 25 aa, synthetic construct
  REGION 1..25: note = FR1
EVQVVESGPELVKPGASVKMSCKTS

SEQ ID NO: 58 - protein, 8 aa, synthetic construct
  REGION 1..8: note = CDR1
AYTFSDSV

SEQ ID NO: 59 - protein, 17 aa, synthetic construct
  REGION 1..17: note = FR2
LSWVKQRTGQGLEWIGE

SEQ ID NO: 60 - protein, 8 aa, synthetic construct
  REGION 1..8: note = CDR2
IYPRGNVT

SEQ ID NO: 61 - protein, 38 aa, synthetic construct
  REGION 1..38: note = FR3
HYNGKFKGKATLTADKSSNTAFMHFSSLTSEDSAVYFC

SEQ ID NO: 62 - protein, 10 aa, synthetic construct
  REGION 1..10: note = CDR3
ARWNNFFFDY

SEQ ID NO: 63 - protein, 11 aa, synthetic construct
  REGION 1..11: note = FR4
WGQGSTLTVSS

SEQ ID NO: 64 - protein, 25 aa, synthetic construct
  REGION 1..25: note = FR1
EVQLQQSGPSLVKPSQTLSLTCSVT

SEQ ID NO: 65 - protein, 8 aa, synthetic construct
  REGION 1..8: note = CDR1
GGSITSFY

SEQ ID NO: 66 - protein, 17 aa, synthetic construct
  REGION 1..17: note = FR2
WNWIRKFPGNKLEYMGY

SEQ ID NO: 67 - protein, 8 aa, synthetic construct
  REGION 1..8: note = CDR2
ISSSGSTY

SEQ ID NO: 68 - protein, 37 aa, synthetic construct
  REGION 1..37: note = FR3
YNPSLKSRISITRDTSKNQSYLQLNSVTAEDTATYYC

SEQ ID NO: 69 - protein, 12 aa, synthetic construct
  REGION 1..12: note = CDR3
ARGGVHYGFGDY

SEQ ID NO: 70 - protein, 11 aa, synthetic construct
  REGION 1..11: note = FR4
WGQGTSVTVSS

SEQ ID NO: 71 - protein, 25 aa, synthetic construct
  REGION 1..25: note = FR1
EVQLVESGGGLVQPGGSLRVSCATS

SEQ ID NO: 72 - protein, 8 aa, synthetic construct
  REGION 1..8: note = CDR1
GFTFSDYY

SEQ ID NO: 73 - protein, 17 aa, synthetic construct
  REGION 1..17: note = FR2
MSWVRQPPGKALEWLGF

SEQ ID NO: 74 - protein, 10 aa, synthetic construct
  REGION 1..10: note = CDR2
IRNKINGYTT

SEQ ID NO: 75 - protein, 38 aa, synthetic construct
  REGION 1..38: note = FR3
EYSASVKGRFTISRDNSQSILYLQMNTLRAEDSATYYC

SEQ ID NO: 76 - protein, 11 aa, synthetic construct
  REGION 1..11: note = CDR3
TRDSSQRPFAY

SEQ ID NO: 77 - protein, 11 aa, synthetic construct
  REGION 1..11: note = FR4
WGQGTLVTVSA

SEQ ID NO: 78 - protein, 25 aa, synthetic construct
  REGION 1..25: note = FR1
EVQLQQSGPELVRPGVSVKISCKGS

SEQ ID NO: 79 - protein, 8 aa, synthetic construct
  REGION 1..8: note = CDR1
GYTFTDYA

SEQ ID NO: 80 - protein, 17 aa, synthetic construct
  REGION 1..17: note = FR2
MHWVKQSHAKSLEWIGV

SEQ ID NO: 81 - protein, 8 aa, synthetic construct
  REGION 1..8: note = CDR2
INTYSGNT

SEQ ID NO: 82 - protein, 38 aa, synthetic construct
  REGION 1..38: note = FR3
YYSQKFKGKATMTVDKSSSTAYMELARLTSEDSAIYYC

SEQ ID NO: 83 - protein, 14 aa, synthetic construct
  REGION 1..14: note = CDR3
ARGAGYFPYWYFDV

SEQ ID NO: 84 - protein, 10 aa, synthetic construct
  REGION 1..10: note = CDR1
GFTFSSYGMS

SEQ ID NO: 85 - protein, 14 aa, synthetic construct
  REGION 1..14: note = FR2
WVRQTPEKRLEWVA

SEQ ID NO: 86 - protein, 17 aa, synthetic construct
  REGION 1..17: note = CDR2
SISGSGSYTYYPDSLKG

SEQ ID NO: 87 - protein, 32 aa, synthetic construct
  REGION 1..32: note = FR3
RFTISRDNAKNNLYLQMSSLRSEDTALYYCAR

SEQ ID NO: 88 - protein, 9 aa, synthetic construct
  REGION 1..9: note = CDR3
QDGYWYFDV

SEQ ID NO: 89 - protein, 25 aa, synthetic construct
  REGION 1..25: note = FR1
EVKLQESGPGLVKPSQSLSLTCTVT

SEQ ID NO: 90 - protein, 9 aa, synthetic construct
  REGION 1..9: note = CDR1
GYSITSDYA

SEQ ID NO: 91 - protein, 18 aa, synthetic construct
  REGION 1..18: note = FR2
WNWIRQFPGNILEWMGYI

SEQ ID NO: 92 - protein, 6 aa, synthetic construct
  REGION 1..6: note = CDR2
SYSGSA

SEQ ID NO: 93 - protein, 38 aa, synthetic construct
  REGION 1..38: note = FR3
SYNPSLQSRISVTRDTSKNQFFLQLNSVTTEDTATYYC

SEQ ID NO: 94 - protein, 12 aa, synthetic construct
  REGION 1..12: note = CDR3
VRSLGRRWYFGF

SEQ ID NO: 95 - protein, 25 aa, synthetic construct
  REGION 1..25: note = FR1
EVQLVESGGGLVKPGGSLKLSCAVS

SEQ ID NO: 96 - protein, 8 aa, synthetic construct
  REGION 1..8: note = CDR1
GFTFSSYA

SEQ ID NO: 97 - protein, 17 aa, synthetic construct
  REGION 1..17: note = FR2
MSWVRQTPEKRLEWVAS

SEQ ID NO: 98 - protein, 7 aa, synthetic construct
  REGION 1..7: note = CDR2
ITDGGIT

SEQ ID NO: 99 - protein, 38 aa, synthetic construct
  REGION 1..38: note = FR3
FYSDSLKGRFTISRDNSGNILYLQMSSLRSEDTAMYFC

SEQ ID NO: 100 - protein, 13 aa, synthetic construct
  REGION 1..13: note = CDR3
ARGSITTDWYFDV

SEQ ID NO: 101 - protein, 8 aa, synthetic construct
  REGION 1..8: note = CDR1
GYTFTDYS

SEQ ID NO: 102 - protein, 8 aa, synthetic construct
  REGION 1..8: note = CDR2
INTSSGNT

SEQ ID NO: 103 - protein, 38 aa, synthetic construct
  REGION 1..38: note = FR3
YYNLKFKGKATMTVDKSSSTAYMELARLTSEDSAIYYC

SEQ ID NO: 104 - protein, 14 aa, synthetic construct
  REGION 1..14: note = CDR3
SKYYGSSFHWYFDV

SEQ ID NO: 105 - protein, 25 aa, synthetic construct
  REGION 1..25: note = FR1
EVQLQQSGPELVRPGESVKISCKGS

SEQ ID NO: 106 - protein, 17 aa, synthetic construct
  REGION 1..17: note = FR2
IHWVKQSHAKSLEWIGV

SEQ ID NO: 107 - protein, 8 aa, synthetic construct
  REGION 1..8: note = CDR2
ISTYYDNT

SEQ ID NO: 108 - protein, 38 aa, synthetic construct
  REGION 1..38: note = FR3
YYNQKFKGRATMTVDKSSSTAYMELARLTSEDSAIYYC

SEQ ID NO: 109 - protein, 14 aa, synthetic construct
  REGION 1..14: note = CDR3
ARGYGSSFNWYFDV

SEQ ID NO: 110 - protein, 25 aa, synthetic construct
  REGION 1..25: note = FR1
EVKLVESGAVLVKPGASVKISCKAS

SEQ ID NO: 111 - protein, 8 aa, synthetic construct
  REGION 1..8: note = CDR1
GYTLSDFN

SEQ ID NO: 112 - protein, 17 aa, synthetic construct
  REGION 1..17: note = FR2
MDWVKQSQGKSLEWVGD

SEQ ID NO: 113 - protein, 8 aa, synthetic construct
  REGION 1..8: note = CDR2
INPNYDTI

SEQ ID NO: 114 - protein, 38 aa, synthetic construct
  REGION 1..38: note = FR3
TYNQKFRGKATLTVDRSSNTAYMELRSLTSEDSAVYYC

SEQ ID NO: 115 - protein, 11 aa, synthetic construct
  REGION 1..11: note = CDR3
ARGELGRYFYV

SEQ ID NO: 116 - protein, 25 aa, synthetic construct
  REGION 1..25: note = FR1
EVQLQQSGAELVQPGASMKLSCKTS

SEQ ID NO: 117 - protein, 8 aa, synthetic construct
  REGION 1..8: note = CDR1
GYTFTTYD

SEQ ID NO: 118 - protein, 17 aa, synthetic construct
  REGION 1..17: note = FR2
INWVRQRPEQGLEWIGW

SEQ ID NO: 119 - protein, 8 aa, synthetic construct
  REGION 1..8: note = CDR2
IFPGDGTT

SEQ ID NO: 120 - protein, 38 aa, synthetic construct
  REGION 1..38: note = FR3
KYNEKFKGKATLTTDKSSSTAYMHLSRLTSEDSVVYFC

SEQ ID NO: 121 - protein, 8 aa, synthetic construct
  REGION 1..8: note = CDR3
ARTPWFDY

SEQ ID NO: 122 - protein, 11 aa, synthetic construct
  REGION 1..11: note = FR4
WGQGTTLTVSS

SEQ ID NO: 123 - protein, 25 aa, synthetic construct
  REGION 1..25: note = FR1
EVQLVESGGGLVKPGGSLRLSCAAS

SEQ ID NO: 124 - protein, 14 aa, synthetic construct
  REGION 1..14: note = FR2
WVRQAPGKGLEWVS

SEQ ID NO: 125 - protein, 32 aa, synthetic construct
  REGION 1..32: note = FR3
RFTISRDNAKNSLYLQMNSLRAEDTAVYYCAR

SEQ ID NO: 126 - protein, 9 aa, synthetic construct
  REGION 1..9: note = CDR3
QQGYWYFDV

SEQ ID NO: 127 - protein, 11 aa, synthetic construct
  REGION 1..11: note = FR4
WGQGTTVTVSS

SEQ ID NO: 128 - protein, 14 aa, synthetic construct
  REGION 1..14: note = FR2
WVRQAPGKRLEWVS

SEQ ID NO: 129 - protein, 14 aa, synthetic construct
  REGION 1..14: note = FR2
WVRQAPGKRLEWVA

SEQ ID NO: 130 - protein, 25 aa, synthetic construct
  REGION 1..25: note = FR1
QVQLVESGAVVKKPGASVKVSCKAS

SEQ ID NO: 131 - protein, 17 aa, synthetic construct
  REGION 1..17: note = FR2
MDWVRQAPGKSLEWMGD

SEQ ID NO: 132 - protein, 38 aa, synthetic construct
  REGION 1..38: note = FR3
TYNQKFRGRVTLTVDRSINTAYMELSRLRSDDTAVYYC

SEQ ID NO: 133 - protein, 11 aa, synthetic construct
  REGION 1..11: note = FR4
WGAGTMVTVSS

SEQ ID NO: 134 - protein, 26 aa, synthetic construct
  REGION 1..26: note = FR1
DIVMTQSPASLAVSLGQRATISCRAS

SEQ ID NO: 135 - protein, 10 aa, synthetic construct
  REGION 1..10: note = CDR1
QSVSTSSYSY

SEQ ID NO: 136 - protein, 17 aa, synthetic construct
  REGION 1..17: note = FR2
MHWYRQIPGQPPKLLIK

SEQ ID NO: 137 - protein, 36 aa, synthetic construct
  REGION 1..36: note = FR3
TLQEGVPSRFSGSGSGTQFTLTISSLQPEDFADYYC

SEQ ID NO: 138 - protein, 36 aa, synthetic construct
  REGION 1..36: note = FR3
NLESGVPARFSGSGSGTDFTLNIHPVEEEDTATYYC

SEQ ID NO: 139 - protein, 9 aa, synthetic construct
  REGION 1..9: note = CDR3
QHSWEIPRT

SEQ ID NO: 140 - protein, 10 aa, synthetic construct
  REGION 1..10: note = FR4
FGGGTKLELK

SEQ ID NO: 141 - protein, 26 aa, synthetic construct
  REGION 1..26: note = FR1
DILMTQTPKFLLVSAGDRVTITCKAS

SEQ ID NO: 142 - protein, 6 aa, synthetic construct
  REGION 1..6: note = CDR1
QSVSND

SEQ ID NO: 143 - protein, 17 aa, synthetic construct
  REGION 1..17: note = FR2
VAWYQQKPGQSPQLLIY

SEQ ID NO: 144 - protein, 36 aa, synthetic construct
  REGION 1..36: note = FR3
HRYTGVPDRFTGSGYGTDFTFTISTVQAEDLAVYFC

SEQ ID NO: 145 - protein, 9 aa, synthetic construct
  REGION 1..9: note = CDR3
QQDNSSPLT

SEQ ID NO: 146 - protein, 10 aa, synthetic construct
  REGION 1..10: note = FR4
FGAGTKLELK

SEQ ID NO: 147 - protein, 26 aa, synthetic construct
  REGION 1..26: note = FR1
DIVMTQPPLSLPVTLGDLASISCRSS

SEQ ID NO: 148 - protein, 11 aa, synthetic construct
  REGION 1..11: note = CDR1
QSLVHSNGITY

SEQ ID NO: 149 - protein, 17 aa, synthetic construct
  REGION 1..17: note = FR2
LHWYLQKPGQSPKLLIY

SEQ ID NO: 150 - protein, 26 aa, synthetic construct
  REGION 1..26: note = FR1
DIQLTQPPSFLSASVGDRVTITCRAS

SEQ ID NO: 151 - protein, 36 aa, synthetic construct [sequence omitted]

SEQ ID NO: 152 - protein, 9 aa, synthetic construct
  REGION 1..9: note = CDR3
SQSTHFPWT

SEQ ID NO: 153 - protein, 26 aa, synthetic construct
  REGION 1..26: note = FR1
DIVMTQSAPSVPVTPGESVSISCRSS

SEQ ID NO: 154 - protein, 11 aa, synthetic construct
  REGION 1..11: note = CDR1
KSLLHSNGNTY

SEQ ID NO: 155 - protein, 17 aa, synthetic construct
  REGION 1..17: note = FR2
LYWFLQRPGQSPQLLIY

SEQ ID NO: 156 - protein, 36 aa, synthetic construct
  REGION 1..36: note = FR3
TLQEGVPSRFSGSGSGTEFTLTISSLQPEDFADYYC

SEQ ID NO: 157 - protein, 36 aa, synthetic construct
  REGION 1..36: note = FR3
NLASGVPDRFSGSGSGTAFTLRISRVEAEDVGVYYC

SEQ ID NO: 158 - protein, 9 aa, synthetic construct
  REGION 1..9: note = CDR3
MQHLEYPLT

SEQ ID NO: 159 - protein, 26 aa, synthetic construct
  REGION 1..26: note = FR1
DIVMTQSPSSLSVSAGEKVTMTCKSS

SEQ ID NO: 160 - protein, 12 aa, synthetic construct
  REGION 1..12: note = CDR1
QSLLNSRSQKNF

SEQ ID NO: 161 - protein, 17 aa, synthetic construct
  REGION 1..17: note = FR2
LAWYQQKPGQPPKLLIY

SEQ ID NO: 162 - protein, 26 aa, synthetic construct
  REGION 1..26: note = FR1
DIQLTQPPSSLSASVGDRVTITCRAS

SEQ ID NO: 163 - protein, 36 aa, synthetic construct
  REGION 1..36: note = FR3
TRESGVPDRFTGSGSGTDFTLTISNVQAEDLAVYYC

SEQ ID NO: 164 - protein, 9 aa, synthetic construct
  REGION 1..9: note = CDR3
QNDLTYPLT

SEQ ID NO: 165 - protein, 26 aa, synthetic construct
  REGION 1..26: note = FR1
DIQMIQSPSYLAASPGETITINCRAS

SEQ ID NO: 166 - protein, 6 aa, synthetic construct
  REGION 1..6: note = CDR1
KSISKY

SEQ ID NO: 167 - protein, 17 aa, synthetic construct
  REGION 1..17: note = FR2
LAWYQEKPGKTNKLLIY

SEQ ID NO: 168 - protein, 17 aa, synthetic construct
  REGION 1..17: note = FR2
LAWYQQKPGRSPQLLVY

SEQ ID NO: 169 - protein, 36 aa, synthetic construct
  REGION 1..36: note = FR3
TLQSGIPSRFSGSGSGTDFTLTISSLEPEDFAMYYC

SEQ ID NO: 170 - protein, 9 aa, synthetic construct
  REGION 1..9: note = CDR3
QQHYEYPYT

SEQ ID NO: 171 - protein, 10 aa, synthetic construct
  REGION 1..10: note = FR4
FGGGTKLEIK

SEQ ID NO: 172 - protein, 23 aa, synthetic construct
  REGION 1..23: note = FR1
DVLMTQTPLSLPVSLGDQVSISC

SEQ ID NO: 173 - protein, 15 aa, synthetic construct
  REGION 1..15: note = CDR1
RASQSLANSYGKTYL

SEQ ID NO: 174 - protein, 16 aa, synthetic construct
  REGION 1..16: note = FR2
SWYLHKPGQSPQLLIY

SEQ ID NO: 175 - protein, 7 aa, synthetic construct
  REGION 1..7: note = CDR2
GISNRFS

SEQ ID NO: 176 - protein, 32 aa, synthetic construct
  REGION 1..32: note = FR3
GVPDRFSGSGSGTDFTLKISTIKPEDLGMYYC

SEQ ID NO: 177 - protein, 9 aa, synthetic construct
  REGION 1..9: note = CDR3
LHGTHQPLT

SEQ ID NO: 178 - protein, 26 aa, synthetic construct
  REGION 1..26: note = FR1
DIVLTQSPSSLAMTVGQKVTMSCKSS

SEQ ID NO: 179 - protein, 12 aa, synthetic construct
  REGION 1..12: note = CDR1
QNLLNSSNQKNY

SEQ ID NO: 180 - protein, 17 aa, synthetic construct
  REGION 1..17: note = FR2
LAWYQQKPGQSPKLLVY

SEQ ID NO: 181 - protein, 36 aa, synthetic construct
  REGION 1..36: note = FR3
TLQEGVPSRFSGSGSGTQFTLTISSLQPEDVADYYC

SEQ ID NO: 182 - protein, 36 aa, synthetic construct
  REGION 1..36: note = FR3
TRESGVPDRFIGSGSGTDFTLTISSVQAEDLADYFC

SEQ ID NO: 183 - protein, 9 aa, synthetic construct
  REGION 1..9: note = CDR3
QQHYSTPLT

SEQ ID NO: 184 - protein, 26 aa, synthetic construct
  REGION 1..26: note = FR1
DIVMTQAPLSLPVSLGDQASISCRSS

SEQ ID NO: 185 - protein, 11 aa, synthetic construct
  REGION 1..11: note = CDR1
QSLVHSNGNTY

SEQ ID NO: 186 - protein, 10 aa, synthetic construct
  REGION 1..10: note = CDR3
SQSTHVPPYT

SEQ ID NO: 187 - protein, 26 aa, synthetic construct
  REGION 1..26: note = FR1
DIVMTQSPVIMSASPGEKVTMTCSAS

SEQ ID NO: 188 - protein, 5 aa, synthetic construct
  REGION 1..5: note = CDR1
SSVSY

SEQ ID NO: 189 - protein, 17 aa, synthetic construct
  REGION 1..17: note = FR2
MHWYQQKSSTSPKLWIY

SEQ ID NO: 190 - protein, 12 aa, synthetic construct
  REGION 1..12: note = FR4
WTFGGGTKVEIK

SEQ ID NO: 191 - protein, 36 aa, synthetic construct
  REGION 1..36: note = FR3
KLASGVPGRFSGTGSGKSHSLTISSMEAEDVATYYC

SEQ ID NO: 192 - protein, 9 aa, synthetic construct
  REGION 1..9: note = CDR3
FQGSGYPLT

SEQ ID NO: 193 - protein, 10 aa, synthetic construct
  REGION 1..10: note = FR4
FGSGTKLEIK

SEQ ID NO: 194 - protein, 26 aa, synthetic construct
  REGION 1..26: note = FR1
DIVMTQSPSSLAVSAGEKVTMSCKSS

SEQ ID NO: 195 - protein, 12 aa, synthetic construct
  REGION 1..12: note = CDR1
QSLLNSRTRKNY

SEQ ID NO: 196 - protein, 17 aa, synthetic construct
  REGION 1..17: note = FR2
LAWYQQKPGQSPKLLIY

SEQ ID NO: 197 - protein, 36 aa, synthetic construct
  REGION 1..36: note = FR3
TLPEGVPSRFSGSGSGTQFTLTISSLQPEDFADYYC

SEQ ID NO: 198 - protein, 36 aa, synthetic construct
  REGION 1..36: note = FR3
TRESGVPDRFTGSGSGTDFTLTITSVQAEDLAVYYC

SEQ ID NO: 199 - protein, 8 aa, synthetic construct
  REGION 1..8: note = CDR3
KQSYNLYT

SEQ ID NO: 200 - protein, 26 aa, synthetic construct
  REGION 1..26: note = FR1
DIQLTQPPASLSASVGETVTITCRAS

SEQ ID NO: 201 - protein, 6 aa, synthetic construct
  REGION 1..6: note = CDR1
ENVYSY

SEQ ID NO: 202 - protein, 17 aa, synthetic construct
  REGION 1..17: note = FR2
LAWYRQKQGRSPQLLVY

SEQ ID NO: 203 - protein, 7 aa, synthetic construct
  REGION 1..7: note = CDR3
SHHYGTP

SEQ ID NO: 204 - protein, 36 aa, synthetic construct
  REGION 1..36: note = FR3
TLPEGVPSRFSGSGSGTQFSLKINSLQTEDLGDYYC

SEQ ID NO: 205 - protein, 7 aa, synthetic construct
  REGION 1..7: note = CDR3
QHHYGTP

SEQ ID NO: 206 - protein, 12 aa, synthetic construct
  REGION 1..12: note = FR4
WTFGGGTKLEIK

SEQ ID NO: 207 - protein, 26 aa, synthetic construct
  REGION 1..26: note = FR1
DIVLSQSPAIMSASPGEKVIMTCSAS

SEQ ID NO: 208 - protein, 5 aa, synthetic construct
  REGION 1..5: note = CDR1
SSISY

SEQ ID NO: 209 - protein, 17 aa, synthetic construct
  REGION 1..17: note = FR2
MYWYQQKPGTSPKRWIY

SEQ ID NO: 210 - protein, 36 aa, synthetic construct
  REGION 1..36: note = FR3
KLASGVPARFSVSGSGTSYSLTISSMEAEDAATYYC

SEQ ID NO: 211 - protein, 8 aa, synthetic construct
  REGION 1..8: note = CDR3
HQRSSYPT

SEQ ID NO: 212 - protein, 23 aa, synthetic construct
  REGION 1..23: note = FR1
DIVMTQTPLSLPVTPGEPASISC

SEQ ID NO: 213 - protein, 15 aa, synthetic construct
  REGION 1..15: note = CDR1
RASQSLASSYGKTYL

SEQ ID NO: 214 - protein, 16 aa, synthetic construct
  REGION 1..16: note = FR2
SWYLQKPGQSPQLLIY

SEQ ID NO: 215 - protein, 32 aa, synthetic construct
  REGION 1..32: note = FR3
GVPDRFSGSGSGTDFTLKISRVEAEDVGVYYC

SEQ ID NO: 216 - protein, 10 aa, synthetic construct
  REGION 1..10: note = FR4
FGQGTKLEIK

SEQ ID NO: 217 - protein, 23 aa, synthetic construct
  REGION 1..23: note = FR1
DVVMTQTPLSLPVTPGEPASISC

SEQ ID NO: 218 - protein, 450 aa, synthetic construct
  REGION 1..450: note = HC
EVQLQQSGTELVRPGALVKLSCKTSGFNIKDCYMHWVKQRPEQGLEWIGWIDPENGNTIYDPKFQGKATITADTSSYTAYLQLSSLTSEDTAVYYCARSRARGYAMDYWGQGTSVTVTSSASTKGPSVFPLAPSSKSTSGGTAALGCLVKDYFPEPVTVSWNSGALTSGVHTFPAVLQSSGLYSLSSVVTVPSSSLGTQTYICNVNHKPSNTKVDKKVEPKSCDKTHTCPPCPAPELLGGPSVFLFPPKPKDTLMISRTPEVTCVVVDVSHEDPEVKFNWYVDGVEVHNAKTKPREEQYNSTYRVVSVLTVLHQDWLNGKEYKCKVSNKALPAPIEKTISKAKGQPREPQVYTLPPSRDELTKNQVSLTCLVKGFYPSDIAVEWESNGQPENNYKTTPPVLDSDGSFFLYSKLTVDKSRWQQGNVFSCSVMHEALHNHYTQKSLSLSPGK

SEQ ID NO: 219 - protein, 218 aa, synthetic construct
  REGION 1..218: note = LC
DIVMTQSPASLAVSLGQRATISCRASQSVSTSSYSYMHWYRQIPGQPPKLLIKYASNLESGVPARFSGSGSGTDFTLNIHPVEEEDTATYYCQHSWEIPRTFGGGTKLELKRTVAAPSVFIFPPSDEQLKSGTASVVCLLNNFYPREAKVQWKVDNALQSGNSQESVTEQDSKDSTYSLSSTLTLSKADYEKHKVYACEVTHQGLSSPVTKSFNRGEC

SEQ ID NO: 220 - protein, 448 aa, synthetic construct
  REGION 1..448: note = HC
EVQLQESGGDLVKPGGSLKLSCAASGFTFSSYGMSWVRQTPEKRLEWVASISGSGSYTYYPDSLKGRFTISRDNAKNNLYLQMSSLRSEDTALYYCARQDGYWYFDVWGAGTTVTVSSASTKGPSVFPLAPSSKSTSGGTAALGCLVKDYFPEPVTVSWNSGALTSGVHTFPAVLQSSGLYSLSSVVTVPSSSLGTQTYICNVNHKPSNTKVDKKVEPKSCDKTHTCPPCPAPELLGGPSVFLFPPKPKDTLMISRTPEVTCVVVDVSHEDPEVKFNWYVDGVEVHNAKTKPREEQYNSTYRVVSVLTVLHQDWLNGKEYKCKVSNKALPAPIEKTISKAKGQPREPQVYTLPPSRDELTKNQVSLTCLVKGFYPSDIAVEWESNGQPENNYKTTPPVLDSDGSFFLYSKLTVDKSRWQQGNVFSCSVMHEALHNHYTQKSLSLSPGK

SEQ ID NO: 221 - protein, 214 aa, synthetic construct
  REGION 1..214: note = LC
DILMTQTPKFLLVSAGDRVTITCKASQSVSNDVAWYQQKPGQSPQLLIYYASHRYTGVPDRFTGSGYGTDFTFTISTVQAEDLAVYFCQQDNSSPLTFGAGTKLELKRTVAAPSVFIFPPSDEQLKSGTASVVCLLNNFYPREAKVQWKVDNALQSGNSQESVTEQDSKDSTYSLSSTLTLSKADYEKHKVYACEVTHQGLSSPVTKSFNRGEC

SEQ ID NO: 222 - protein, 447 aa, synthetic construct
  REGION 1..447: note = HC
EVQVVESGPELVKPGASVKMSCKTSAYTFSDSVLSWVKQRTGQGLEWIGEIYPRGNVTHYNGKFKGKATLTADKSSNTAFMHFSSLTSEDSAVYFCARWNNFFFDYWGQGSTLTVSSASTKGPSVFPLAPSSKSTSGGTAALGCLVKDYFPEPVTVSWNSGALTSGVHTFPAVLQSSGLYSLSSVVTVPSSSLGTQTYICNVNHKPSNTKVDKKVEPKSCDKTHTCPPCPAPELLGGPSVFLFPPKPKDTLMISRTPEVTCVVVDVSHEDPEVKFNWYVDGVEVHNAKTKPREEQYNSTYRVVSVLTVLHQDWLNGKEYKCKVSNKALPAPIEKTISKAKGQPREPQVYTLPPSRDELTKNQVSLTCLVKGFYPSDIAVEWESNGQPENNYKTTPPVLDSDGSFFLYSKLTVDKSRWQQGNVFSCSVMHEALHNHYTQKSLSLSPGK

SEQ ID NO: 223 - protein, 219 aa, synthetic construct
  REGION 1..219: note = LC
DIVMTQPPLSLPVTLGDLASISCRSSQSLVHSNGITYLHWYLQKPGQSPKLLIYKVSNRFSGVPDRFSGSGSGTDFTLKISRVEAEDLGVYFCSQSTHFPWTFGGGTKLELKRTVAAPSVFIFPPSDEQLKSGTASVVCLLNNFYPREAKVQWKVDNALQSGNSQESVTEQDSKDSTYSLSSTLTLSKADYEKHKVYACEVTHQGLSSPVTKSFNRGEC

SEQ ID NO: 224 - protein, 448 aa, synthetic construct
  REGION 1..448: note = HC
EVQLQQSGPSLVKPSQTLSLTCSVTGGSITSFYWNWIRKFPGNKLEYMGYISSSGSTYYNPSLKSRISITRDTSKNQSYLQLNSVTAEDTATYYCARGGVHYGFGDYWGQGTSVTVSSASTKGPSVFPLAPSSKSTSGGTAALGCLVKDYFPEPVTVSWNSGALTSGVHTFPAVLQSSGLYSLSSVVTVPSSSLGTQTYICNVNHKPSNTKVDKKVEPKSCDKTHTCPPCPAPELLGGPSVFLFPPKPKDTLMISRTPEVTCVVVDVSHEDPEVKFNWYVDGVEVHNAKTKPREEQYNSTYRVVSVLTVLHQDWLNGKEYKCKVSNKALPAPIEKTISKAKGQPREPQVYTLPPSRDELTKNQVSLTCLVKGFYPSDIAVEWESNGQPENNYKTTPPVLDSDGSFFLYSKLTVDKSRWQQGNVFSCSVMHEALHNHYTQKSLSLSPGK

SEQ ID NO: 225 - protein, 219 aa, synthetic construct
  REGION 1..219: note = LC
DIVMTQSAPSVPVTPGESVSISCRSSKSLLHSNGNTYLYWFLQRPGQSPQLLIYRMSNLASGVPDRFSGSGSGTAFTLRISRVEAEDVGVYYCMQHLEYPLTFGAGTKLELKRTVAAPSVFIFPPSDEQLKSGTASVVCLLNNFYPREAKVQWKVDNALQSGNSQESVTEQDSKDSTYSLSSTLTLSKADYEKHKVYACEVTHQGLSSPVTKSFNRGEC

SEQ ID NO: 226 - protein, 450 aa, synthetic construct
  REGION 1..450: note = HC
EVQLVESGGGLVQPGGSLRVSCATSGFTFSDYYMSWVRQPPGKALEWLGFIRNKINGYTTEYSASVKGRFTISRDNSQSILYLQMNTLRAEDSATYYCTRDSSQRPFAYWGQGTLVTVSAASTKGPSVFPLAPSSKSTSGGTAALGCLVKDYFPEPVTVSWNSGALTSGVHTFPAVLQSSGLYSLSSVVTVPSSSLGTQTYICNVNHKPSNTKVDKKVEPKSCDKTHTCPPCPAPELLGGPSVFLFPPKPKDTLMISRTPEVTCVVVDVSHEDPEVKFNWYVDGVEVHNAKTKPREEQYNSTYRVVSVLTVLHQDWLNGKEYKCKVSNKALPAPIEKTISKAKGQPREPQVYTLPPSRDELTKNQVSLTCLVKGFYPSDIAVEWESNGQPENNYKTTPPVLDSDGSFFLYSKLTVDKSRWQQGNVFSCSVMHEALHNHYTQKSLSLSPGK

SEQ ID NO: 227 - protein, 220 aa, synthetic construct
  REGION 1..220: note = LC
DIVMTQSPSSLSVSAGEKVTMTCKSSQSLLNSRSQKNFLAWYQQKPGQPPKLLIYGASTRESGVPDRFTGSGSGTDFTLTISNVQAEDLAVYYCQNDLTYPLTFGAGTKLELKRTVAAPSVFIFPPSDEQLKSGTASVVCLLNNFYPREAKVQWKVDNALQSGNSQESVTEQDSKDSTYSLSSTLTLSKADYEKHKVYACEVTHQGLSSPVTKSFNRGEC

SEQ ID NO: 228 - protein, 451 aa, synthetic construct
  REGION 1..451: note = HC
EVQLQQSGPELVRPGVSVKISCKGSGYTFTDYAMHWVKQSHAKSLEWIGVINTYSGNTYYSQKFKGKATMTVDKSSSTAYMELARLTSEDSAIYYCARGAGYFPYWYFDVWGAGTTVTVSSASTKGPSVFPLAPSSKSTSGGTAALGCLVKDYFPEPVTVSWNSGALTSGVHTFPAVLQSSGLYSLSSVVTVPSSSLGTQTYICNVNHKPSNTKVDKKVEPKSCDKTHTCPPCPAPELLGGPSVFLFPPKPKDTLMISRTPEVTCVVVDVSHEDPEVKFNWYVDGVEVHNAKTKPREEQYNSTYRVVSVLTVLHQDWLNGKEYKCKVSNKALPAPIEKTISKAKGQPREPQVYTLPPSRDELTKNQVSLTCLVKGFYPSDIAVEWESNGQPENNYKTTPPVLDSDGSFFLYSKLTVDKSRWQQGNVFSCSVMHEALHNHYTQKSLSLSPGK

SEQ ID NO: 229 - protein, 214 aa, synthetic construct
  REGION 1..214: note = LC
DIQMIQSPSYLAASPGETITINCRASKSISKYLAWYQEKPGKTNKLLIYSGSTLQSGIPSRFSGSGSGTDFTLTISSLEPEDFAMYYCQQHYEYPYTFGGGTKLEIKRTVAAPSVFIFPPSDEQLKSGTASVVCLLNNFYPREAKVQWKVDNALQSGNSQESVTEQDSKDSTYSLSSTLTLSKADYEKHKVYACEVTHQGLSSPVTKSFNRGEC

SEQ ID NO: 230 - protein, 448 aa, synthetic construct; identical to SEQ ID NO: 220
  REGION 1..448: note = HC

SEQ ID NO: 231 - protein, 219 aa, synthetic construct
  REGION 1..219: note = LC
DVLMTQTPLSLPVSLGDQVSISCRASQSLANSYGKTYLSWYLHKPGQSPQLLIYGISNRFSGVPDRFSGSGSGTDFTLKISTIKPEDLGMYYCLHGTHQPLTFGAGTKLELKRTVAAPSVFIFPPSDEQLKSGTASVVCLLNNFYPREAKVQWKVDNALQSGNSQESVTEQDSKDSTYSLSSTLTLSKADYEKHKVYACEVTHQGLSSPVTKSFNRGEC

SEQ ID NO: 232 - protein, 449 aa, synthetic construct
  REGION 1..449: note = HC
EVKLQESGPGLVKPSQSLSLTCTVTGYSITSDYAWNWIRQFPGNILEWMGYISYSGSASYNPSLQSRISVTRDTSKNQFFLQLNSVTTEDTATYYCVRSLGRRWYFGFWGAGTTVTVSSASTKGPSVFPLAPSSKSTSGGTAALGCLVKDYFPEPVTVSWNSGALTSGVHTFPAVLQSSGLYSLSSVVTVPSSSLGTQTYICNVNHKPSNTKVDKKVEPKSCDKTHTCPPCPAPELLGGPSVFLFPPKPKDTLMISRTPEVTCVVVDVSHEDPEVKFNWYVDGVEVHNAKTKPREEQYNSTYRVVSVLTVLHQDWLNGKEYKCKVSNKALPAPIEKTISKAKGQPREPQVYTLPPSRDELTKNQVSLTCLVKGFYPSDIAVEWESNGQPENNYKTTPPVLDSDGSFFLYSKLTVDKSRWQQGNVFSCSVMHEALHNHYTQKSLSLSPGK

SEQ ID NO: 233 - protein, 220 aa, synthetic construct
  REGION 1..220: note = LC
DIVLTQSPSSLAMTVGQKVTMSCKSSQNLLNSSNQKNYLAWYQQKPGQSPKLLVYFASTRESGVPDRFIGSGSGTDFTLTISSVQAEDLADYFCQQHYSTPLTFGGGTKLEIKRTVAAPSVFIFPPSDEQLKSGTASVVCLLNNFYPREAKVQWKVDNALQSGNSQESVTEQDSKDSTYSLSSTLTLSKADYEKHKVYACEVTHQGLSSPVTKSFNRGEC

SEQ ID NO: 234 - protein, 449 aa, synthetic construct
  REGION 1..449: note = HC
EVQLVESGGGLVKPGGSLKLSCAVSGFTFSSYAMSWVRQTPEKRLEWVASITDGGITFYSDSLKGRFTISRDNSGNILYLQMSSLRSEDTAMYFCARGSITTDWYFDVWGAGTTVTVSSASTKGPSVFPLAPSSKSTSGGTAALGCLVKDYFPEPVTVSWNSGALTSGVHTFPAVLQSSGLYSLSSVVTVPSSSLGTQTYICNVNHKPSNTKVDKKVEPKSCDKTHTCPPCPAPELLGGPSVFLFPPKPKDTLMISRTPEVTCVVVDVSHEDPEVKFNWYVDGVEVHNAKTKPREEQYNSTYRVVSVLTVLHQDWLNGKEYKCKVSNKALPAPIEKTISKAKGQPREPQVYTLPPSRDELTKNQVSLTCLVKGFYPSDIAVEWESNGQPENNYKTTPPVLDSDGSFFLYSKLTVDKSRWQQGNVFSCSVMHEALHNHYTQKSLSLSPGK

SEQ ID NO: 235 - protein, 220 aa, synthetic construct
  REGION 1..220: note = LC
DIVMTQAPLSLPVSLGDQASISCRSSQSLVHSNGNTYLHWYLQKPGQSPKLLIYKVSNRFSGVPDRFSGSGSGTDFTLKISRVEAEDLGVYFCSQSTHVPPYTFGGGTKLEIKRTVAAPSVFIFPPSDEQLKSGTASVVCLLNNFYPREAKVQWKVDNALQSGNSQESVTEQDSKDSTYSLSSTLTLSKADYEKHKVYACEVTHQGLSSPVTKSFNRGEC

SEQ ID NO: 236 - protein, 451 aa, synthetic construct
  REGION 1..451: note = HC
EVQLQQSGPELVRPGVSVKISCKGSGYTFTDYSMHWVKQSHAKSLEWIGVINTSSGNTYYNLKFKGKATMTVDKSSSTAYMELARLTSEDSAIYYCSKYYGSSFHWYFDVWGAGTTVTVSSASTKGPSVFPLAPSSKSTSGGTAALGCLVKDYFPEPVTVSWNSGALTSGVHTFPAVLQSSGLYSLSSVVTVPSSSLGTQTYICNVNHKPSNTKVDKKVEPKSCDKTHTCPPCPAPELLGGPSVFLFPPKPKDTLMISRTPEVTCVVVDVSHEDPEVKFNWYVDGVEVHNAKTKPREEQYNSTYRVVSVLTVLHQDWLNGKEYKCKVSNKALPAPIEKTISKAKGQPREPQVYTLPPSRDELTKNQVSLTCLVKGFYPSDIAVEWESNGQPENNYKTTPPVLDSDGSFFLYSKLTVDKSRWQQGNVFSCSVMHEALHNHYTQKSLSLSPGK

SEQ ID NO: 237 - protein, 213 aa, synthetic construct
  REGION 1..213: note = LC
DIVMTQSPVIMSASPGEKVTMTCSASSSVSYMHWYQQKSSTSPKLWIYDTSKLASGVPGRFSGTGSGKSHSLTISSMEAEDVATYYCFQGSGYPLTFGSGTKLEIKRTVAAPSVFIFPPSDEQLKSGTASVVCLLNNFYPREAKVQWKVDNALQSGNSQESVTEQDSKDSTYSLSSTLTLSKADYEKHKVYACEVTHQGLSSPVTKSFNRGEC

SEQ ID NO: 238 - protein, 451 aa, synthetic construct
  REGION 1..451: note = HC
EVQLQQSGPELVRPGESVKISCKGSGYTFTDYAIHWVKQSHAKSLEWIGVISTYYDNTYYNQKFKGRATMTVDKSSSTAYMELARLTSEDSAIYYCARGYGSSFNWYFDVWGAGTTVTVSSASTKGPSVFPLAPSSKSTSGGTAALGCLVKDYFPEPVTVSWNSGALTSGVHTFPAVLQSSGLYSLSSVVTVPSSSLGTQTYICNVNHKPSNTKVDKKVEPKSCDKTHTCPPCPAPELLGGPSVFLFPPKPKDTLMISRTPEVTCVVVDVSHEDPEVKFNWYVDGVEVHNAKTKPREEQYNSTYRVVSVLTVLHQDWLNGKEYKCKVSNKALPAPIEKTISKAKGQPREPQVYTLPPSRDELTKNQVSLTCLVKGFYPSDIAVEWESNGQPENNYKTTPPVLDSDGSFFLYSKLTVDKSRWQQGNVFSCSVMHEALHNHYTQKSLSLSPGK

SEQ ID NO: 239 - protein, 219 aa, synthetic construct
  REGION 1..219: note = LC
DIVMTQSPSSLAVSAGEKVTMSCKSSQSLLNSRTRKNYLAWYQQKPGQSPKLLIYWASTRESGVPDRFTGSGSGTDFTLTITSVQAEDLAVYYCKQSYNLYTFGGGTKLEIKRTVAAPSVFIFPPSDEQLKSGTASVVCLLNNFYPREAKVQWKVDNALQSGNSQESVTEQDSKDSTYSLSSTLTLSKADYEKHKVYACEVTHQGLSSPVTKSFNRGEC

SEQ ID NO: 240 - protein, 448 aa, synthetic construct
  REGION 1..448: note = HC
EVKLVESGAVLVKPGASVKISCKASGYTLSDFNMDWVKQSQGKSLEWVGDINPNYDTITYNQKFRGKATLTVDRSSNTAYMELRSLTSEDSAVYYCARGELGRYFYVWGAGTTVTVSSASTKGPSVFPLAPSSKSTSGGTAALGCLVKDYFPEPVTVSWNSGALTSGVHTFPAVLQSSGLYSLSSVVTVPSSSLGTQTYICNVNHKPSNTKVDKKVEPKSCDKTHTCPPCPAPELLGGPSVFLFPPKPKDTLMISRTPEVTCVVVDVSHEDPEVKFNWYVDGVEVHNAKTKPREEQYNSTYRVVSVLTVLHQDWLNGKEYKCKVSNKALPAPIEKTISKAKGQPREPQVYTLPPSRDELTKNQVSLTCLVKGFYPSDIAVEWESNGQPENNYKTTPPVLDSDGSFFLYSKLTVDKSRWQQGNVFSCSVMHEALHNHYTQKSLSLSPGK

SEQ ID NO: 241 - protein, 214 aa, synthetic construct
  REGION 1..214: note = LC
DIQLTQPPASLSASVGETVTITCRASENVYSYLAWYRQKQGRSPQLLVYNAKTLPEGVPSRFSGSGSGTQFSLKINSLQTEDLGDYYCQHHYGTPWTFGGGTKLEIKRTVAAPSVFIFPPSDEQLKSGTASVVCLLNNFYPREAKVQWKVDNALQSGNSQESVTEQDSKDSTYSLSSTLTLSKADYEKHKVYACEVTHQGLSSPVTKSFNRGEC

SEQ ID NO: 242 - protein, 445 aa, synthetic construct
  REGION 1..445: note = HC
EVQLQQSGAELVQPGASMKLSCKTSGYTFTTYDINWVRQRPEQGLEWIGWIFPGDGTTKYNEKFKGKATLTTDKSSSTAYMHLSRLTSEDSVVYFCARTPWFDYWGQGTTLTVSSASTKGPSVFPLAPSSKSTSGGTAALGCLVKDYFPEPVTVSWNSGALTSGVHTFPAVLQSSGLYSLSSVVTVPSSSLGTQTYICNVNHKPSNTKVDKKVEPKSCDKTHTCPPCPAPELLGGPSVFLFPPKPKDTLMISRTPEVTCVVVDVSHEDPEVKFNWYVDGVEVHNAKTKPREEQYNSTYRVVSVLTVLHQDWLNGKEYKCKVSNKALPAPIEKTISKAKGQPREPQVYTLPPSRDELTKNQVSLTCLVKGFYPSDIAVEWESNGQPENNYKTTPPVLDSDGSFFLYSKLTVDKSRWQQGNVFSCSVMHEALHNHYTQKSLSLSPGK

SEQ ID NO: 243 - protein, 212 aa, synthetic construct
  REGION 1..212: note = LC
DIVLSQSPAIMSASPGEKVIMTCSASSSISYMYWYQQKPGTSPKRWIYDTSKLASGVPARFSVSGSGTSYSLTISSMEAEDAATYYCHQRSSYPTFGGGTKLELKRTVAAPSVFIFPPSDEQLKSGTASVVCLLNNFYPREAKVQWKVDNALQSGNSQESVTEQDSKDSTYSLSSTLTLSKADYEKHKVYACEVTHQGLSSPVTKSFNRGEC

SEQ ID NO: 244 - protein, 448 aa, synthetic construct
  REGION 1..448: note = HC
EVQLQQSGPELVRPGVSVKISCKGSGYTFTDYAMHWVRQSHAKSLECIGVINTYSGNTNYNQKFKGKATMTVDRSSSTAYMELARLTSEDSAIYYCARVYGNYPYWYFDVWGAGTTVTASTKGPSVFPLAPSSKSTSGGTAALGCLVKDYFPEPVTVSWNSGALTSGVHTFPAVLQSSGLYSLSSVVTVPSSSLGTQTYICNVNHKPSNTKVDKKVEPKSCDKTHTCPPCPAPELLGGPSVFLFPPKPKDTLMISRTPEVTCVVVDVSHEDPEVKFNWYVDGVEVHNAKTKPREEQYNSTYRVVSVLTVLHQDWLNGKEYKCKVSNKALPAPIEKTISKAKGQPREPQVYTLPPSRDELTKNQVSLTCLVKGFYPSDIAVEWESNGQPENNYKTTPPVLDSDGSFFLYSKLTVDKSRWQQGNVFSCSVMHEALHNHYTQKSLSLSPGK

SEQ ID NO: 245 - protein, 213 aa, synthetic construct
  REGION 1..213: note = LC
DILMTQSPAIMSASPGEKVTMTCRASSSVSSSYLHWYQQKSGASPKLWIYSTSNLASGVPARFSGSGSGTSYSLTISSVEAEDAATYYCQQYSGYPLTFGAGTKLERTVAAPSVFIFPPSDEQLKSGTASVVCLLNNFYPREAKVQWKVDNALQSGNSQESVTEQDSKDSTYSLSSTLTLSKADYEKHKVYACEVTHQGLSSPVTKSFNRGEC

SEQ ID NO: 246 - protein, 450 aa, synthetic construct
  REGION 1..450: note = HC
EVQLQQSGAELVKPRASVRLSCRASGYTFTSYWMHWVKQRPGQGLEWIGMIHPNSGSTNYNEKFKSKATLTVDKSSSTAYMQLSSLTSEDSAVYFCARERFGLLRYFDYWGQGTTLTVSSASTKGPSVFPLAPSSKSTSGGTAALGCLVKDYFPEPVTVSWNSGALTSGVHTFPAVLQSSGLYSLSSVVTVPSSSLGTQTYICNVNHKPSNTKVDKKVEPKSCDKTHTCPPCPAPELLGGPSVFLFPPKPKDTLMISRTPEVTCVVVDVSHEDPEVKFNWYVDGVEVHNAKTKPREEQYNSTYRVVSVLTVLHQDWLNGKEYKCKVSNKALPAPIEKTISKAKGQPREPQVYTLPPSRDELTKNQVSLTCLVKGFYPSDIAVEWESNGQPENNYKTTPPVLDSDGSFFLYSKLTVDKSRWQQGNVFSCSVMHEALHNHYTQKSLSLSPGK

SEQ ID NO: 247 - protein, 214 aa, synthetic construct
  REGION 1..214: note = LC
DIVMTQSPSSMYASLGERVTITCKASQDINSFLSWFQQKPGKSPKTLLYRANRLMDGVPSRFSGSGSGQDFSLTISSREYEDMGIYYCLQYDEFPFTFGSGTKLELKRTVAAPSVFIFPPSDEQLKSGTASVVCLLNNFYPREAKVQWKVDNALQSGNSQESVTEQDSKDSTYSLSSTLTLSKADYEKHKVYACEVTHQGLSSPVTKSFNRGEC

SEQ ID NO: 248 - protein, 448 aa, synthetic construct
  REGION 1..448: note = HC
EVQLVESGGGLVKPGGSLRLSCAASGFTFSSYGMSWVRQAPGKGLEWVSSISGSGSYTYYPDSLKGRFTISRDNAKNSLYLQMNSLRAEDTAVYYCARQQGYWYFDVWGQGTTVTVSSASTKGPSVFPLAPSSKSTSGGTAALGCLVKDYFPEPVTVSWNSGALTSGVHTFPAVLQSSGLYSLSSVVTVPSSSLGTQTYICNVNHKPSNTKVDKRVEPKSCDKTHTCPPCPAPELLGGPSVFLFPPKPKDTLMISRTPEVTCVVVDVSHEDPEVKFNWYVDGVEVHNAKTKPREEQYNSTYRVVSVLTVLHQDWLNGKEYKCKVSNKALPAPIEKTISKAKGQPREPQVYTLPPSREEMTKNQVSLTCLVKGFYPSDIAVEWESNGQPENNYKTTPPVLDSDGSFFLYSKLTVDKSRWQQGNVFSCSVMHEALHNHYTQKSLSLSPGK

SEQ ID NO: 249 - protein, 219 aa, synthetic construct
  REGION 1..219: note = LC
DIVMTQTPLSLPVTPGEPASISCRASQSLASSYGKTYLSWYLQKPGQSPQLLIYGISNRFSGVPDRFSGSGSGTDFTLKISRVEAEDVGVYYCLHGTHQPLTFGQGTKLEIKRTVAAPSVFIFPPSDEQLKSGTASVVCLLNNFYPREAKVQWKVDNALQSGNSQESVTEQDSKDSTYSLSSTLTLSKADYEKHKVYACEVTHQGLSSPVTKSFNRGEC

SEQ ID NO: 250 - protein, 448 aa, synthetic construct
  REGION 1..448: note = HC
EVQLVESGGGLVKPGGSLRLSCAASGFTFSSYGMSWVRQAPGKRLEWVSSISGSGSYTYYPDSLKGRFTISRDNAKNSLYLQMNSLRAEDTAVYYCARQQGYWYFDVWGQGTTVTVSSASTKGPSVFPLAPSSKSTSGGTAALGCLVKDYFPEPVTVSWNSGALTSGVHTFPAVLQSSGLYSLSSVVTVPSSSLGTQTYICNVNHKPSNTKVDKRVEPKSCDKTHTCPPCPAPELLGGPSVFLFPPKPKDTLMISRTPEVTCVVVDVSHEDPEVKFNWYVDGVEVHNAKTKPREEQYNSTYRVVSVLTVLHQDWLNGKEYKCKVSNKALPAPIEKTISKAKGQPREPQVYTLPPSREEMTKNQVSLTCLVKGFYPSDIAVEWESNGQPENNYKTTPPVLDSDGSFFLYSKLTVDKSRWQQGNVFSCSVMHEALHNHYTQKSLSLSPGK

SEQ ID NO: 251 - protein, 219 aa, synthetic construct
  REGION 1..219: note = LC
DVVMTQTPLSLPVTPGEPASISCRASQSLASSYGKTYLSWYLQKPGQSPQLLIYGISNRFSGVPDRFSGSGSGTDFTLKISRVEAEDVGVYYCLHGTHQPLTFGQGTKLEIKRTVAAPSVFIFPPSDEQLKSGTASVVCLLNNFYPREAKVQWKVDNALQSGNSQESVTEQDSKDSTYSLSSTLTLSKADYEKHKVYACEVTHQGLSSPVTKSFNRGEC

SEQ ID NO: 252 - protein, 448 aa, synthetic construct
  REGION 1..448: note = HC
EVQLVESGGGLVKPGGSLRLSCAASGFTFSSYGMSWVRQAPGKRLEWVASISGSGSYTYYPDSLKGRFTISRDNAKNSLYLQMNSLRAEDTAVYYCARQQGYWYFDVWGQGTTVTVSSASTKGPSVFPLAPSSKSTSGGTAALGCLVKDYFPEPVTVSWNSGALTSGVHTFPAVLQSSGLYSLSSVVTVPSSSLGTQTYICNVNHKPSNTKVDKRVEPKSCDKTHTCPPCPAPELLGGPSVFLFPPKPKDTLMISRTPEVTCVVVDVSHEDPEVKFNWYVDGVEVHNAKTKPREEQYNSTYRVVSVLTVLHQDWLNGKEYKCKVSNKALPAPIEKTISKAKGQPREPQVYTLPPSREEMTKNQVSLTCLVKGFYPSDIAVEWESNGQPENNYKTTPPVLDSDGSFFLYSKLTVDKSRWQQGNVFSCSVMHEALHNHYTQKSLSLSPGK

SEQ ID NO: 253 - protein, 448 aa, synthetic construct
  REGION 1..448: note = HC
EVQLQESGGDLVKPGGSLKLSCAASGFTFSSYGMSWVRQTPEKRLEWVASISGSGSYTYYPDSLKGRFTISRDNAKNNLYLQMSSLRSEDTALYYCARQDGYWYFDVWGAGTTVTVSSASTKGPSVFPLAPSSKSTSGGTAALGCLVKDYFPEPVTVSWNSGALTSGVHTFPAVLQSSGLYSLSSVVTVPSSSLGTQTYICNVNHKPSNTKVDKRVEPKSCDKTHTCPPCPAPELLGGPSVFLFPPKPKDTLMISRTPEVTCVVVDVSHEDPEVKFNWYVDGVEVHNAKTKPREEQYNSTYRVVSVLTVLHQDWLNGKEYKCKVSNKALPAPIEKTISKAKGQPREPQVYTLPPSREEMTKNQVSLTCLVKGFYPSDIAVEWESNGQPENNYKTTPPVLDSDGSFFLYSKLTVDKSRWQQGNVFSCSVMHEALHNHYTQKSLSLSPGK

SEQ ID NO: 254 - protein, 219 aa, synthetic construct; identical to SEQ ID NO: 231
  REGION 1..219: note = LC

SEQ ID NO: 255 - protein, 448 aa, synthetic construct
  REGION 1..448: note = HC
EVKLVESGAVLVKPGASVKISCKASGYTLSDFNMDWVKQSQGKSLEWVGDINPNYDTITYNQKFRGKATLTVDRSSNTAYMELRSLTSEDSAVYYCARGELGRYFYVWGAGTTVTVSSASTKGPSVFPLAPSSKSTSGGTAALGCLVKDYFPEPVTVSWNSGALTSGVHTFPAVLQSSGLYSLSSVVTVPSSSLGTQTYICNVNHKPSNTKVDKRVEPKSCDKTHTCPPCPAPELLGGPSVFLFPPKPKDTLMISRTPEVTCVVVDVSHEDPEVKFNWYVDGVEVHNAKTKPREEQYNSTYRVVSVLTVLHQDWLNGKEYKCKVSNKALPAPIEKTISKAKGQPREPQVYTLPPSREEMTKNQVSLTCLVKGFYPSDIAVEWESNGQPENNYKTTPPVLDSDGSFFLYSKLTVDKSRWQQGNVFSCSVMHEALHNHYTQKSLSLSPGK

SEQ ID NO: 256 - protein, 448 aa, synthetic construct
  REGION 1..448: note = HC
QVQLVESGAVVKKPGASVKVSCKASGYTLSDFNMDWVRQAPGKSLEWMGDINPNYDTITYNQKFRGRVTLTVDRSINTAYMELSRLRSDDTAVYYCARGELGRYFYVWGAGTMVTVSSASTKGPSVFPLAPSSKSTSGGTAALGCLVKDYFPEPVTVSWNSGALTSGVHTFPAVLQSSGLYSLSSVVTVPSSSLGTQTYICNVNHKPSNTKVDKRVEPKSCDKTHTCPPCPAPELLGGPSVFLFPPKPKDTLMISRTPEVTCVVVDVSHEDPEVKFNWYVDGVEVHNAKTKPREEQYNSTYRVVSVLTVLHQDWLNGKEYKCKVSNKALPAPIEKTISKAKGQPREPQVYTLPPSREEMTKNQVSLTCLVKGFYPSDIAVEWESNGQPENNYKTTPPVLDSDGSFFLYSKLTVDKSRWQQGNVFSCSVMHEALHNHYTQKSLSLSPGK

SEQ ID NO: 257 - protein, 448 aa, synthetic construct
  REGION 1..448: note = HC
EVQLVESGAVVKKPGASVKVSCKASGYTLSDFNMDWVRQAPGKSLEWMGDINPNYDTITYNQKFRGRVTLTVDRSANTAYMELSSLRSEDTAVYYCARGELGRYFYVWGAGTMVTVSSASTKGPSVFPLAPSSKSTSGGTAALGCLVKDYFPEPVTVSWNSGALTSGVHTFPAVLQSSGLYSLSSVVTVPSSSLGTQTYICNVNHKPSNTKVDKRVEPKSCDKTHTCPPCPAPELLGGPSVFLFPPKPKDTLMISRTPEVTCVVVDVSHEDPEVKFNWYVDGVEVHNAKTKPREEQYNSTYRVVSVLTVLHQDWLNGKEYKCKVSNKALPAPIEKTISKAKGQPREPQVYTLPPSREEMTKNQVSLTCLVKGFYPSDIAVEWESNGQPENNYKTTPPVLDSDGSFFLYSKLTVDKSRWQQGNVFSCSVMHEALHNHYTQKSLSLSPGK

SEQ ID NO: 258 - protein, 448 aa, synthetic construct
  REGION 1..448: note = HC
EVKLVESGAEVKKPGASVKVSCKASGYTLSDFNMDWVRQAPGKSLEWMGDINPNYDTITYNQKFRGRVTLTVDRSTNTAYMELSSLRSEDTAVYYCARGELGRYFYVWGAGTMVTVSSASTKGPSVFPLAPSSKSTSGGTAALGCLVKDYFPEPVTVSWNSGALTSGVHTFPAVLQSSGLYSLSSVVTVPSSSLGTQTYICNVNHKPSNTKVDKRVEPKSCDKTHTCPPCPAPELLGGPSVFLFPPKPKDTLMISRTPEVTCVVVDVSHEDPEVKFNWYVDGVEVHNAKTKPREEQYNSTYRVVSVLTVLHQDWLNGKEYKCKVSNKALPAPIEKTISKAKGQPREPQVYTLPPSREEMTKNQVSLTCLVKGFYPSDIAVEWESNGQPENNYKTTPPVLDSDGSFFLYSKLTVDKSRWQQGNVFSCSVMHEALHNHYTQKSLSLSPGK

SEQ ID NO: 259 - protein, 448 aa, synthetic construct
  REGION 1..448: note = HC
QVQLVESGAEVKKPGASVKVSCKASGYTLSDFNMDWVRQAQGKSLEWMGDINPNYDTITYNQKFRGRVTLTVDRSTNTAYMELSSLRSEDTAVYYCARGELGRYFYVWGAGTMVTVSSASTKGPSVFPLAPSSKSTSGGTAALGCLVKDYFPEPVTVSWNSGALTSGVHTFPAVLQSSGLYSLSSVVTVPSSSLGTQTYICNVNHKPSNTKVDKRVEPKSCDKTHTCPPCPAPELLGGPSVFLFPPKPKDTLMISRTPEVTCVVVDVSHEDPEVKFNWYVDGVEVHNAKTKPREEQYNSTYRVVSVLTVLHQDWLNGKEYKCKVSNKALPAPIEKTISKAKGQPREPQVYTLPPSREEMTKNQVSLTCLVKGFYPSDIAVEWESNGQPENNYKTTPPVLDSDGSFFLYSKLTVDKSRWQQGNVFSCSVMHEALHNHYTQKSLSLSPGK

SEQ ID NO: 260 - protein, 214 aa, synthetic construct
  REGION 1..214: note = LC
DIQLTQPPSSLSASVGDRVTITCRASENVYSYLAWYQQKPGRSPQLLVYNAKTLQEGVPSRFSGSGSGTQFTLTISSLQPEDFADYYCQHHYGTPWTFGGGTKVEIKRTVAAPSVFIFPPSDEQLKSGTASVVCLLNNFYPREAKVQWKVDNALQSGNSQESVTEQDSKDSTYSLSSTLTLSKADYEKHKVYACEVTHQGLSSPVTKSFNRGEC

SEQ ID NO: 261 - protein, 214 aa, synthetic construct; identical to SEQ ID NO: 260
  REGION 1..214: note = LC

SEQ ID NO: 262 - protein, 214 aa, synthetic construct
  REGION 1..214: note = LC
DIQLTQPPSFLSASVGDRVTITCRASENVYSYLAWYQQKPGRSPQLLVYNAKTLQEGVPSRFSGSGSGTEFTLTISSLQPEDFADYYCQHHYGTPWTFGGGTKVEIKRTVAAPSVFIFPPSDEQLKSGTASVVCLLNNFYPREAKVQWKVDNALQSGNSQESVTEQDSKDSTYSLSSTLTLSKADYEKHKVYACEVTHQGLSSPVTKSFNRGEC

SEQ ID NO: 263 - protein, 214 aa, synthetic construct
  REGION 1..214: note = LC
DIQLTQPPSSLSASVGDRVTITCRASENVYSYLAWYQQKPGRSPQLLVYNAKTLQEGVPSRFSGSGSGTQFTLTISSLQPEDVADYYCQHHYGTPWTFGGGTKVEIKRTVAAPSVFIFPPSDEQLKSGTASVVCLLNNFYPREAKVQWKVDNALQSGNSQESVTEQDSKDSTYSLSSTLTLSKADYEKHKVYACEVTHQGLSSPVTKSFNRGEC

SEQ ID NO: 264 - protein, 214 aa, synthetic construct
  REGION 1..214: note = LC
DIQLTQPPSSLSASVGDRVTITCRASENVYSYLAWYQQKPGRSPQLLVYNAKTLPEGVPSRFSGSGSGTQFTLTISSLQPEDFADYYCSHHYGTPWTFGGGTKVEIKRTVAAPSVFIFPPSDEQLKSGTASVVCLLNNFYPREAKVQWKVDNALQSGNSQESVTEQDSKDSTYSLSSTLTLSKADYEKHKVYACEVTHQGLSSPVTKSFNRGEC

SEQ ID NO: 265 - protein, 118 aa, synthetic construct
  REGION 1..118: note = VH
EVQLQQSGPELVRPGVSVKISCKGSGYTFTDYAMHWVRQSHAKSLECIGVINTYSGNTNYNQKFKGKATMTVDRSSSTAYMELARLTSEDSAIYYCARVYGNYPYWYFDVWGAGTTVT

SEQ ID NO: 266 - protein, 106 aa, synthetic construct
  REGION 1..106: note = VL
DILMTQSPAIMSASPGEKVTMTCRASSSVSSSYLHWYQQKSGASPKLWIYSTSNLASGVPARFSGSGSGTSYSLTISSVEAEDAATYYCQQYSGYPLTFGAGTKLE

SEQ ID NO: 267 - protein, 120 aa, synthetic construct
  REGION 1..120: note = VH
EVQLQQSGAELVKPRASVRLSCRASGYTFTSYWMHWVKQRPGQGLEWIGMIHPNSGSTNYNEKFKSKATLTVDKSSSTAYMQLSSLTSEDSAVYFCARERFGLLRYFDYWGQGTTLTVSS

SEQ ID NO: 268 - protein, 107 aa, synthetic construct
  REGION 1..107: note = VL
DIVMTQSPSSMYASLGERVTITCKASQDINSFLSWFQQKPGKSPKTLLYRANRLMDGVPSRFSGSGSGQDFSLTISSREYEDMGIYYCLQYDEFPFTFGSGTKLELK

SEQ ID NO: 269 - protein, 450 aa, synthetic construct
  REGION 1..450: note = HC
QVQLVQSGAEVKKPGSSVKVSCKASGYTFTNYVMHWVRQAPGQGLEWMGYINPYNDDVKYNEKFKGRVTITADESTSTAYMELSSLRSEDTAVYYCARWGYYGSPLYYFDYWGQGTLVTVSSASTKGPSVFPLAPSSKSTSGGTAALGCLVKDYFPEPVTVSWNSGALTSGVHTFPAVLQSSGLYSLSSVVTVPSSSLGTQTYICNVNHKPSNTKVDKRVEPKSCDKTHTCPPCPAPELLGGPSVFLFPPKPKDTLMISRTPEVTCVVVDVSHEDPEVKFNWYVDGVEVHNAKTKPREEQYNSTYRVVSVLTVLHQDWLNGKEYKCKVSNKALPAPIEKTISKAKGQPREPQVYTLPPSREEMTKNQVSLTCLVKGFYPSDIAVEWESNGQPENNYKTTPPVLDSDGSFFLYSKLTVDKSRWQQGNVFSCSVMHEALHNHYTQKSLSLSP

SEQ ID NO: 270 - protein, 213 aa, synthetic construct
  REGION 1..213: note = LC
EIVLTQSPATLSLSPGERATLSCRASSRLIYMHWYQQKPGQAPRPLIYATSNLASGIPARFSGSGSGTDFTLTISSLEPEDFAVYYCQQWNSNPPTFGQGTKVEIKRTVAAPSVFIFPPSDEQLKSGTASVVCLLNNFYPREAKVQWKVDNALQSGNSQESVTEQDSKDSTYSLSSTLTLSKADYEKHKVYACEVTHQGLSSPVTKSFNRGEC

SEQ ID NO: 271 - protein, 447 aa, synthetic construct
  REGION 1..447: note = HC
EVQLVESGGGLVKPGGSLRLSCAASGFTFSSYGMSWVRQAPGKGLEWVATINSGGSNTYYPDSLKGRFTISRDNAKNSLYLQMNSLRAEDTAVYYCARHDGGAMDYWGQGTTVTVSSASTKGPSVFPLAPSSKSTSGGTAALGCLVKDYFPEPVTVSWNSGALTSGVHTFPAVLQSSGLYSLSSVVTVPSSSLGTQTYICNVNHKPSNTKVDKRVEPKSCDKTHTCPPCPAPELLGGPSVFLFPPKPKDTLMISRTPEVTCVVVDVSHEDPEVKFNWYVDGVEVHNAKTKPREEQYNSTYRVVSVLTVLHQDWLNGKEYKCKVSNKALPAPIEKTISKAKGQPREPQVYTLPPSREEMTKNQVSLTCLVKGFYPSDIAVEWESNGQPENNYKTTPPVLDSDGSFFLYSKLTVDKSRWQQGNVFSCSVMHEALHNHYTQKSLSLSPGK

SEQ ID NO: 272 - protein, 215 aa, synthetic construct
  REGION 1..215: note = LC
DIQMTQSPSSLSASVGDRVTITCRASESIYSYLAWYQQKPGKAPKLLVYNTKTLPEGVPSRFSGSGSGTDFTLTISSLQPEDFATYYCQHHYGTPPWTFGQGTRLEIKRTVAAPSVFIFPPSDEQLKSGTASVVCLLNNFYPREAKVQWKVDNALQSGNSQESVTEQDSKDSTYSLSSTLTLSKADYEKHKVYACEVTHQGLSSPVTKSFNRGEC